European Patent Application EP 4 707 380 A1, published March 11, 2026. Title: Lactobacillus mali strain and uses thereof. Applicant: CJ CheilJedang Corporation. Application KR. The sequence listing filed with the application follows.

SEQUENCE LISTING (1 sequence)

SEQ ID NO: 1 - DNA, 1209 bp, synthetic construct
  misc_feature 1..1209: note = Lactobacillus mali CJST01 27F 16S rRNA sequence
  source 1..1209: mol_type = other DNA
tgcggtggcggcagctatacatgcagtcgaacgcaaaactttcatcgaatgcttgcattcaccgaaagttttgagtggcgaacgggtgagtaacacgtgggtaacctgcccagaagagggggataacacttggaaacaggtgctaataccgcataacaataaaaaccgcatggtttttatttaaaagatggttttgctatcacttctggatggacccgcggcgtattagctagttggtaaggtaaaggcttaccaaggcaatgatacgtagccgaactgagaggttgatcggccacattgggactgagacacggcccaaactcctacgggaggcagcagtagggaatcttccacaatggacgaaagtctgatggagcaacgccgcgtgagtgaagaaggttttcggatcgtaaaactctgttgttagagaagaacgtgtgtgagagtaactgctcatgcagtgacggtatctaaccagaaagccacggctaactacgtgccagcagccgcggtaatacgtaggtggcaagcgttgtccggatttattgggcgtaaagggaacgcaggcggttttttaagtctgatgtgaaagccttcggcttaaccgaagtcatgcattggaaactgaaagacttgagtgcagaagaggagagtggaactccatgtgtagcggtgaaatgcgtagatatatggaagaacaccagtggcgaaagcggctctctggtctgtaactgacgctgaggttcgaaagtgtgggtagcaaacaggattagataccctggtagtccacaccgtaaacgatgaatgctaagtgttggagggtttccgcccttcggtgctgcagctaacgcattaagcattccgcctggggagtacgaccgcaaggttgaaactcaaaggaattgacgggggcccgcacaagcggtggagcatgtggtttaattcgaagcaacgcgaagaacccttaccaggtcttgacatcttctgacaaccctaagagattagtgttccctttcgggacagaatgacaggtggtgcatgatgtcgtcagctcgtgtcgtgagatgttgggttaagtcccgcacgagcgcactctatatagttgcagcatagtgggcactctagtgagactggcgtgacaacgaggagtgggatgacgtcaatcatcatgcccctaatgaaccttggggcttaaacacacacggtgtc